European Patent Specification EP 3 361 869 B1, published December 3, 2025. Title: NUCLEIC ACID MOLECULES CONTAINING SPACERS AND METHODS OF USE THEREOF. Applicant: Audentes Therapeutics, Inc. The sequence listing filed with the application follows.

SEQUENCE LISTING (12 sequences)

SEQ ID NO: 1 - DNA, 3000 bp, Homo sapiens
gtaaaaaaaggcatagctaacaaggtgtggaaaaagaattagtggttagagagtgagctattcgttgaaacaattgcgttcttgaaacaattcttgctggtaaaatgtcacattttatgtgactacaggtggaggattggcacataacctaaccagtgggggaaacaattgacctctggatttgtccaagtgtatagtagcatttgcccaatcgaatggtcctggtaaggtgttaatgttgactagaaccaaaggtggaagttgcagggaaactggtttagtacaagggtggacaccaggcagtcatccagaggcccattaaaggccttggaatgtttttccgaaggagaatcactccctcttctctcgcttaaagttttaggggattcatgaacagctgctgtgggatagtttcatgtccctagcaattgtaaagcaactgagggtggcttaaaccagttttagctttagggttagggttactggactaaaatttgagaaattcataaatcttaaggaaatccattgtgagttttcattatgagtgcatccaatgtataatttccatgaccctcccatgcaagtgagcatgtgaatcaggaaacgttacaagaacccaacaaactcaaccactactagacaggcgatcacttccagttagtatgcaactttctgtgtaattttagttaccattaaaatctggatgaccttagtgtaaggaaaaaataccttgaatagtgttaaagatgtacacttggtgtcaggcattgtaacattgataaatctgtgtaaggtgctttttgaaaacttcaaagctgcatcaagtcaagtacaagaaaggccatggctgctaaagctgttgaagatgtgggatggaactgggtcacattggtgttaacagcgttgtgcagagccggcaggatcttggtgtgagcgaacattagtctatttaataaagctgtgtgaatgttgtagaggtgaggatgctcacttgaaaactcactgaagaacacttggccccttgaactaaagtgcttctatcaagttcagtgagaaattccgaattacaagcataggtactagaaaagttttgaaaagcagtatagagcaacataagcacattcataaaattagtgatgtagaaagtgaaatttccacgtatggtcactcccagagaaaaaaaatacgtttatttaccttttttaaaaataggggatttcaggccgggtgaggtggctcacgcctgtaatcccagcactttgggaggcccaggtgggcggatcacctgaggtcaggagttggagggatggcaaatcccatctctacaaaatatacaaaaaaatagctgggtgtgttggcaggcgcctgtaatcccagctactcggaaggctgaggcaggagaatccctggaaccagggatgtggaggttgcagtgagccgagattgtgtaactgcattccagcctgggcaacaagagcaagactccgtatcaggaaaaaaaaaagggggggttggatttcgcttgttgcataggttggtctcaaactcctggcctcaagtgattctcctgcctctgcctcccaaagtgctgagattacaggtgtgaggcaccatgccaggtctcttactgtttgtaattaaatacatacacattttgtgtgtttgtgtgcacctttataaagtcaaaggtgatagtaacccatttaagttcctactcaattttactttccagggataactaactactttttctttttgagatggagtctcgctgtgtagcccaggctggagtgcagtggcaccatctcggctcactgcaagctcctcctccctggttcacgctattctcctgcctcagcctccccaacaactaggactacaggctcacctcgccatacctggctaattttttgtatttttagtagagacagggtttcactgtgttagccaggatggtctcgatctcctgaccttgtgatccgcctgcctctgcctcccaaagtgctgggattacaggcatgagcaacctcacccagctgggataactactttttacaggttgatattcttttggacttttcccctgtgtaaaaatatactatatttgttatgtacatattatgtacatacagacacaaattggaccattctcagtataatgattctcaggttttttttttttttttgaggtggggaactagataattatggacatctttccatactagcatatcaatatctacctcattctttttaatatttttgctagtattccattgtatgaatgtcctatgatttacttaacctgtccatcaatatttgtttccaggtttttgctattataatgctgctgcaaagtacatcctcacacatctttattttgtctattcatatttctgtaagataggttactaaagttggaactgccaaattaacactatcatactattttgttttttaattttaattttttaaaaaatgtaaaatgtgcaatttcaagaggagaaacttgaacacaaggagcaaaatctatttttataacatcctattaaaagcttgctttacataaagattttgaaagaatagcataaatacaagatttctattttaattggattcttagggctaataaaataatcagccttagcacttatttatttattttttttgagagggagtctcgctctgttgtccatgctggagtgcagtggcgtgatctcggctcactgcaagctccacctcatgagttcacaccattctcctgcctcagtctcccgagtagctgggactccaggcgccctctacaaagcccgtctaattttttttgtatttttagtagagacagggtttcactgtgttagccaggatggtcttgatctcctgaccttgtgatctgcccgcctcggcctcccaaagtgctgggattataggcttgagccactgctcccggccagcacttatttttataattcttcatgattactgtgttactgtcccatg

SEQ ID NO: 2 - DNA, 2884 bp, Homo sapiens
atatttctcaatttttaaatttttcaaaaaaattaatccttaatgtgcatatttttgaattgttaatataactttttgaggtgatgtcttcatgtgtttcaactacttaaaaacttttaaacagtatataataaaaaatcttccaggccactcacacctgtaatcccagcactttgggaggctgaggtgggcagatcacctgagggcaggagttcgagaccagcctggccaatatatatatattcatatattcatatatatatatatattcatatattcatatatatatattcatatattcatatatatatatatatatatatatagcaaaacctcatctctaataaaatacaaaaattagctgagcgtggtgatggatgcctgtagtcccagctactcgggaggctgaggcaggagaatctcttgaacctgggaggtggaggttgcagtgagctgagatggtgccactgccctccagcctgagtgacagagcgagactcggtctccaaaaaaaaacaacaaaaaaatcttccatccttgtctcccatccaccccttccccccagcatgtacttgcagactttatgcatatacagtgagtactgtatatacacaaataataaaaaaatcatatatataatatatgtaattcccctttacatgaaaggtagcacactggtctgtacagtctgtctgcactgtgctatttcactttatatttttatagtttgacagagttctaacatttctttttttttttttttaacagagtcttgttcctgattgttaaattttaaagcatcctaaagtttggtttcacacttgaatgaataccatgtaaggattcacttacatagatgtggttgcctgaatcttaagaataaaataacattgtttgtatttatttaaattagtgttccttttatggtttgcctgaaagcacaacaaaatcctcaccaagatattacaattatgactcccatacaggtaaactgtttagagattggcaagcaccttttaatgaaaggagtcagccagcttagtgtgcagtatttatttctgccggaagagggagcttcagggacagactttggtttagtcatgaagcctccagcactcccaagcggttgtggttgaccaagcaatttatgcttttacctttctacttccagaggcttgtttacttatcagtaagcattaatttagtgtcccctcagatgccttttactttcttcttttctgcctagaataagctgctcttccaattttgcagctacatgtttccaccccagttggaatttctccataacatccattgtagctatccttcaatctacagcctctatttcctgttatagctggtcaggtctaatccctcaaaatactctgtcccctgcttcccttatctgctggccacctttttcccccacatacacactgccatgtcccacccttcactcaagttgttccctgccacctcaacaaatttaagtccataaaatagagtaagtgttcctgactgttaaattttaaagcatcccaaagtctgatttcacactcgaatgaatactatgtacggattcatttacatagatgcggttgcatgagtcttaacaaaaaaataacattatttgtatttattcaaagtactgtcaagatataatgtcaagacctaattcaaaggttccacaaagccttccttgactgcccccaacgaagattatccattttccctgaaatcccattgacttttctattttgtaaggaggctcgtgagactctgtctaaaaacaaaacaaaacaaaaagaaacaatcaaacggcttgcttctgttctttgatctgctagtaagcaaaaattacacatggtgacaggagctatgtgaggctgtcaggttgaatgggaggagtttgggatcctgcttgtggatggttggaagaggctttcgggaaagacagtatttatgtgagacctggaagatgggccttagctttgcagaaggtggagaggcaggaaatagcacgggggccctggggctggaagacttgggcatatttgaggaacagaaaggagaccagcataactgaggtgggaaaagcatgtgaagagatggggctggaggaggccgggagtggtggctcacgcctgtaatcccagcactttgggaggccaaggcaggcggatcatgagctcaggagattgagaccatcctggctaacacggtgaaaccccctctctactaaaaatacaaaaaaaaaaaaaaaaaaaattagctgggcgtggtggcaggagcctgtagtcccagctacctgggaggctgaggcaggagaatggcgtgaacctggaaggctgagcttgcagtgagccgagattgcaccactgcactccagcctgggagacagagagagactccctctcaaaaaaacaaacaaacgaaacaaaacaaaacaaaaattagccaggcgtggtggtatgcacctgtaatcccagctactcgggaggttgaggcaggagaaacgcttgaactcaggaggcggaggttgcagtgagccgagactgcgccactgcactccagcctcaacctccccagctgaagccatcctcttgcctcagcctcctaagtagctgggactacaggcgcgcacctccaggcttggctcttattctttttattgtttttgaaactatagaacctatttttaaaaaatgttttggttgtttttattgctgcttttccttttggggttagaacacaagttttgatgggaaacaggttagaacacattcatctcttcccatagcgatggtcatagaaaaacggggcatatttataaactctcagttgatcttaaaatgtgcaaaagctgccgaactcctgggagtga

SEQ ID NO: 3 - DNA, 1501 bp, Homo sapiens
gaaaagggggggttggatttcgcttgttgcataggttggtctcaaactcctggcctcaagtgattctcctgcctctgcctcccaaagtgctgagattacaggtgtgaggcaccatgccaggtctcttactgtttgtaattaaatacatacacattttgtgtgtttgtgtgcacctttataaagtcaaaggtgatagtaacccatttaagttcctactcaattttactttccagggataactaactactttttctttttgagatggagtctcgctgtgtagcccaggctggagtgcagtggcaccatctcggctcactgcaagctcctcctccctggttcacgctattctcctgcctcagcctccccaacaactaggactacaggctcacctcgccatacctggctaattttttgtatttttagtagagacagggtttcactgtgttagccaggatggtctcgatctcctgaccttgtgatccgcctgcctctgcctcccaaagtgctgggattacaggcatgagcaacctcacccagctgggataactactttttacaggttgatattcttttggacttttcccctgtgtaaaaatatactatatttgttatgtacatattatgtacatacagacacaaattggaccattctcagtataatgattctcaggttttttttttttttttgaggtggggaactagataattatggacatctttccatactagcatatcaatatctacctcattctttttaatatttttgctagtattccattgtatgaatgtcctatgatttacttaacctgtccatcaatatttgtttccaggtttttgctattataatgctgctgcaaagtacatcctcacacatctttattttgtctattcatatttctgtaagataggttactaaagttggaactgccaaattaacactatcatactattttgttttttaattttaattttttaaaaaatgtaaaatgtgcaatttcaagaggagaaacttgaacacaaggagcaaaatctatttttataacatcctattaaaagcttgctttacataaagattttgaaagaatagcataaatacaagatttctattttaattggattcttagggctaataaaataatcagccttagcacttatttatttattttttttgagagggagtctcgctctgttgtccatgctggagtgcagtggcgtgatctcggctcactgcaagctccacctcatgagttcacaccattctcctgcctcagtctcccgagtagctgggactccaggcgccctctacaaagcccgtctaattttttttgtatttttagtagagacagggtttcactgtgttagccaggatggtcttgatctcctgaccttgtgatctgcccgcctcggcctcccaaagtgctgggattataggcttgagccactgctcccggccagcacttatttttataattcttcatgattactgtgttactgtcccatg

SEQ ID NO: 4 - DNA, 1501 bp, Homo sapiens
atatttctcaatttttaaatttttcaaaaaaattaatccttaatgtgcatatttttgaattgttaatataactttttgaggtgatgtcttcatgtgtttcaactacttaaaaacttttaaacagtatataataaaaaatcttccaggccactcacacctgtaatcccagcactttgggaggctgaggtgggcagatcacctgagggcaggagttcgagaccagcctggccaatatatatatattcatatattcatatatatatatatattcatatattcatatatatatattcatatattcatatatatatatatatatatatatagcaaaacctcatctctaataaaatacaaaaattagctgagcgtggtgatggatgcctgtagtcccagctactcgggaggctgaggcaggagaatctcttgaacctgggaggtggaggttgcagtgagctgagatggtgccactgccctccagcctgagtgacagagcgagactcggtctccaaaaaaaaacaacaaaaaaatcttccatccttgtctcccatccaccccttccccccagcatgtacttgcagactttatgcatatacagtgagtactgtatatacacaaataataaaaaaatcatatatataatatatgtaattcccctttacatgaaaggtagcacactggtctgtacagtctgtctgcactgtgctatttcactttatatttttatagtttgacagagttctaacatttctttttttttttttttaacagagtcttgttcctgattgttaaattttaaagcatcctaaagtttggtttcacacttgaatgaataccatgtaaggattcacttacatagatgtggttgcctgaatcttaagaataaaataacattgtttgtatttatttaaattagtgttccttttatggtttgcctgaaagcacaacaaaatcctcaccaagatattacaattatgactcccatacaggtaaactgtttagagattggcaagcaccttttaatgaaaggagtcagccagcttagtgtgcagtatttatttctgccggaagagggagcttcagggacagactttggtttagtcatgaagcctccagcactcccaagcggttgtggttgaccaagcaatttatgcttttacctttctacttccagaggcttgtttacttatcagtaagcattaatttagtgtcccctcagatgccttttactttcttcttttctgcctagaataagctgctcttccaattttgcagctacatgtttccaccccagttggaatttctccataacatccattgtagctatccttcaatctacagcctctatttcctgttatagctggtcaggtctaatccctcaaaatactctgtcccctgcttcccttatctgctggccacctttttcccccacatacacactgccatgtcccacccttcactcaagttgttccctgccacctcaacaaatttaagtccataaaac

SEQ ID NO: 5 - DNA, 14 bp, Homo sapiens
gagcgagcgagcgc

SEQ ID NO: 6 - DNA, 6015 bp, Homo sapiens
gagggtttcagcgctaaaactaggctgtcctgggcaaacagcataagctggtcaccccacacccagacctgacccaaacccagctcccctgcttcttggccacgtaacctgagaagggaatccctcctctctgaaccccagcccaccccaatgctccaggcctcctgggataccccgaagagtgagtttgccaagcagtcaccccacagttggaggagaatccacccaaaaggcagcctggtagacagggctggggtggcctctcgtggggtccaggccaagtaggtggcctggggcctctgggggatgcaggggaagggggatgcaggggaacggggatgcaggggaacggggctcagtctgaagagcagagccaggaacccctgtagggaaggggcaggagagccaggggcatgagatggtggacgaggaagggggacagggaagcctgagcgcctctcctgggcttgccaaggactcaaacccagaagcccagagcagggccttagggaagcgggaccctgctctgggcggaggaatatgtcccagatagcactggggactctttaaggaaagaaggatggagaaagagaaagggagtagaggcggccacgacctggtgaacacctaggacgcaccattctcacaaagggagttttccacacggacacccccctcctcaccacagccctgccaggacggggctggctactggccttatctcacaggtaaaactgacgcacggaggaacaatataaattggggactagaaaggtgaagagccaaagttagaactcaggaccaacttattctgattttgtttttccaaactgcttctcctcttgggaagtgtaaggaagctgcagcaccaggatcagtgaaacgcaccagacagccgcgtcagagcagctcaggttctgggagagggtagcgcagggtggccactgagaaccgggcaggtcacgcatcccccccttccctcccaccccctgccaagctctccctcccaggatcctctctggctccatcgtaagcaaaccttagaggttctggcaaggagagagatggctccaggaaatgggggtgtgtcaccagataaggaatctgcctaacaggaggtgggggttagacccaatatcaggagactaggaaggaggaggcctaaggatggggcttttctgtcaccaatcctgtccctagtggccccactgtggggtggaggggacagataaaagtacccagaaccagagccacattaaccggccctgggaatataaggtggtcccagctcggggacacaggatccctggaggcagcaaacatgctgtcctgaagtggacataggggcccgggttggaggaagaagactagctgagctctcggacccctggaagatgccatgacagggggctggaagagctagcacagactagagaggtaaggggggtaggggagctgcccaaatgaaaggagtgagaggtgacccgaatccacaggagaacggggtgtccaggcaaagaaagcaagaggatggagaggtggctaaagccagggagacggggtactttggggttgtccagaaaaacggtgatgatgcaggcctacaagaaggggaggcgggacgcaagggagacatccgtcggagaaggccatcctaagaaacgagagatggcacaggccccagaaggagaaggaaaagggaacccagcgagtgaagacggcatggggttgggtgagggaggagagatgcccggagaggacccagacacggggaggatccgctcagaggacatcacgtggtgcagcgccgagaaggaagtgctccggaaagagcatccttgggcagcaacacagcagagagcaaggggaagagggagtggaggaagacggaacctgaaggaggcggcagggaaggatctgggccagccgtagaggtgacccaggccacaagctgcagacagaaagcggcacaggcccaggggagagaatgcaggtcagagaaagcaggacctgcctgggaaggggaaacagtgggccagaggcggcgcagaagccagtagagctcaaagtggtccggactcaggagagagacggcagcgttagagggcagagttccggcggcacagcaagggcactcgggggcgagaggagggcagcgcaaagtgacaatggccagggccaggcagatagaccagactgagctatgggagctggctcaggttcaggagagggcagggcagggaaggagacaaagtccaggaccggctggaggggctcaacatcggaagaggggaagtcgagggagggatggtaaggaggactgcatgggtcagcacaggctgccaaagccagggccagttaaagcgactccaatgcggaagagagtaggtcgaaggggaatggtaaggaggcctggggcagagtggtcagcacagagtggctaagcccagggccagttgaagcggctccaattcggaagtggggtggtcgaaggggaatggtaagggggactgggacggggtgtcagcatagggtggcaaagcccagggccaggaacgacggggcggatcgagactggcaacggggaaggaggatgccccaggtggcgcagcagagggtggacctggccccgggagacgccgggcggggggcgctgacctggtgcagggcgctgataccgtcggcgttggtggagtccagcacggcgcgggcgggcggcggcgcggcggggtcgagctcggcgccggggccagggtcggcggcgcgcagcatcagacgcgcctcgtccaggtcgccgcccgcacaggccgccaggaactcggcggcgcgctcgaagcggacggtgcgggcgcggcgctctccggggccaggctcggcgcccgcccgcgccccccactgccgcagctgctcccgtcgccgctcccgggcagccgccgccgccgcccccgggccagccgccgggccatcctctccggacatcgcaccgcccgcccgcccagcgagcgagcgagcgccgagccccaaccgccgccaccacccgcccgcccgcccgccccgggggccgccgggaactgccgctggccccccaccgccccaaggatctcccggtccccgcccggcgtgctgacgtcacggcgctgccccagggtgtgctgggcaggtcgcggggagcgctgggaaatggagtccattagcagaagtggcccttggccacttccaggagtcgctgtgccccgatgcacactgggaagtccgcagctccgaggcgcccagtggaaatcgccagatgagggcctcctccggggaatgctgggaaatggagtctacaggccggaggggtgccccacggcatactaggaagtgtgtagcaccgggtaaaggggatgaatagcagactgccccggggcagttaggaattcgactggacagccgcgtgggagggagtgcggggagaggcagagttgttttgttattgttgttttattttgttttctttgttttgagacggagtctcgctctgtcgccacgctggagttcagtggcgcgatatcggctcgctgcaacctccgcttcccaggttcaagcaattctggctcagtccccagagtagctgggataacaggcgcgcgccaccccgccctgctaatttttatatttttagtagagacgggatttcaccatgttggccatgatggtcttgatctcttgacctcatgatccgcccgcctcggcctgtaatcctgctgggatgacgagcgtaagccaccatgcccagctgggttttatttattttggtttttttcctgaccccttaactagaaataagctccacgagagcgggatcttttgtcttctgtgcactacttgtcctcggttcttagaacagaacctgagagaacctgatcgcaaatatttttggaatgaatgaatgaatgggttcaccagggcaccatgggaaactgagtccgcaacctagaagccatgaaagacagtccacttccaagcttccctgggtgacctcgcagggcatgctgggaaatgaaatttgcggtgaaaaggtcaggaccacgatcctagggcacgctgggaaatgtagcccacagggccacacccctaaaagcacagtggggtgcaaggcagggccccaaggcatttagggctcggggcaagagaaatccacactccactccctaatggtaatccctgagccacaccgagtaaaggaacccaagacacagtgtccacagggacagggctctcagagctttcactggcccgcgcttctcctgcgcccacccggacctcctgggaaccgcccaggccctcgcgcgctctcaaggcatgctgggattggtggtcccgggcaaggagttccagcaggtggggggcgaatcacctttcagcgggcccaagcgatgagcacaccttgatcttcaccttacggatcccgcgcccaactcaagattgggaaggtggctggcactttgtgacaggaagagtcccataaaaatcatacagaaaagggccaaaatcgggacagagactacagactgtttcccaagcgctgtgggagtttcccacccactctgaagtccttgggtttgcgcggagacgtaaactgcgcatcccacgaggcctgtttctttccctctctctttctcttttgttgttgttgttgctgctgctgttacgaaaatttttgtggttttattgtatcatgaggcattgaaacatccggcgactcaatgtctaggcggtgaggcagccgctttctccttcactttctttgggttaagtagagcaacttgtcagtagttttgtttttttttgttgttgttgttgtttttgagacggaggcttgctctgtcgcccaggctggagtgcagtggcgcgatgtcggctcactgcaagctctgcctcccgggttcaagcgattctcctgcctcagcctcctgagtagctgggactacaggcgtgctccaccacgcccggctaatttttgttttttagtagagacggggtttcaccatgttggccaggctggtctcgaattcctgacctcgtgatccgactgcctcggcctcccaaaatgctgggattacaggcgtgagccgccgcgaccggccagattttttttttttttaaaggacaaccttttgcattacttaagtctttccaaggcatgcgctggtacaacacaaacttttcccattacatgcagctagtctagtgtccagacgtcatgcacaacacctccgtggcatcagcgcactgcgcccactcccactgcgaccctgctcatttgtgcatcatatctggaggagtggcaatagttctggaaagaggagggaagaggaggcagcgtgagggcccggtggagaggaggtcagctgaagttgtgcagagcaagcctgcatatcattggtgcaaacccaagcatcattgcatcgctgatgttttgttttgtttggttttgttttgtttttgagacggagtctcactgtgtcgcccaggctggagtgcagtgatgtgatctcggctcactgcaacctccgcctcccaggttcaagtgattctcctacctcagcctcccaagtagctgggattacaggcgtgctccacgcctggctaatttttgtatttttagtagagacaaggtttcaccatgttggccaggctggtctcgatctcctgacctcaagtgatccacccgcctcagcttcccaaagtgctgggattacaggcatgagccaccacacccagctgatgttctttagtaggaatatctggtggaaccccaagatggggtcttcatccgccacgaagcctgtttctatagaaagggatagttctggtggctcttaggtgtggtccctgaaccccacactttccacatacttacacaccaacctccttcccccaggaaaacaagaagtcggtcttcagggtgttaccgtgtagctctggttctgtatgtattctgtgcctttatgtataattgtgtgtatttgcaat

SEQ ID NO: 7 - DNA, 3000 bp, Homo sapiens
catgggacagtaacacagtaatcatgaagaattataaaaataagtgctggccgggagcagtggctcaagcctataatcccagcactttgggaggccgaggcgggcagatcacaaggtcaggagatcaagaccatcctggctaacacagtgaaaccctgtctctactaaaaatacaaaaaaaattagacgggctttgtagagggcgcctggagtcccagctactcgggagactgaggcaggagaatggtgtgaactcatgaggtggagcttgcagtgagccgagatcacgccactgcactccagcatggacaacagagcgagactccctctcaaaaaaaataaataaataagtgctaaggctgattattttattagccctaagaatccaattaaaatagaaatcttgtatttatgctattctttcaaaatctttatgtaaagcaagcttttaataggatgttataaaaatagattttgctccttgtgttcaagtttctcctcttgaaattgcacattttacattttttaaaaaattaaaattaaaaaacaaaatagtatgatagtgttaatttggcagttccaactttagtaacctatcttacagaaatatgaatagacaaaataaagatgtgtgaggatgtactttgcagcagcattataatagcaaaaacctggaaacaaatattgatggacaggttaagtaaatcataggacattcatacaatggaatactagcaaaaatattaaaaagaatgaggtagatattgatatgctagtatggaaagatgtccataattatctagttccccacctcaaaaaaaaaaaaaaaacctgagaatcattatactgagaatggtccaatttgtgtctgtatgtacataatatgtacataacaaatatagtatatttttacacaggggaaaagtccaaaagaatatcaacctgtaaaaagtagttatcccagctgggtgaggttgctcatgcctgtaatcccagcactttgggaggcagaggcaggcggatcacaaggtcaggagatcgagaccatcctggctaacacagtgaaaccctgtctctactaaaaatacaaaaaattagccaggtatggcgaggtgagcctgtagtcctagttgttggggaggctgaggcaggagaatagcgtgaaccagggaggaggagcttgcagtgagccgagatggtgccactgcactccagcctgggctacacagcgagactccatctcaaaaagaaaaagtagttagttatccctggaaagtaaaattgagtaggaacttaaatgggttactatcacctttgactttataaaggtgcacacaaacacacaaaatgtgtatgtatttaattacaaacagtaagagacctggcatggtgcctcacacctgtaatctcagcactttgggaggcagaggcaggagaatcacttgaggccaggagtttgagaccaacctatgcaacaagcgaaatccaacccccccttttttttttcctgatacggagtcttgctcttgttgcccaggctggaatgcagttacacaatctcggctcactgcaacctccacatccctggttccagggattctcctgcctcagccttccgagtagctgggattacaggcgcctgccaacacacccagctatttttttgtatattttgtagagatgggatttgccatccctccaactcctgacctcaggtgatccgcccacctgggcctcccaaagtgctgggattacaggcgtgagccacctcacccggcctgaaatcccctatttttaaaaaaggtaaataaacgtattttttttctctgggagtgaccatacgtggaaatttcactttctacatcactaattttatgaatgtgcttatgttgctctatactgcttttcaaaacttttctagtacctatgcttgtaattcggaatttctcactgaacttgatagaagcactttagttcaaggggccaagtgttcttcagtgagttttcaagtgagcatcctcacctctacaacattcacacagctttattaaatagactaatgttcgctcacaccaagatcctgccggctctgcacaacgctgttaacaccaatgtgacccagttccatcccacatcttcaacagctttagcagccatggcctttcttgtacttgacttgatgcagctttgaagttttcaaaaagcaccttacacagatttatcaatgttacaatgcctgacaccaagtgtacatctttaacactattcaaggtattttttccttacactaaggtcatccagattttaatggtaactaaaattacacagaaagttgcatactaactggaagtgatcgcctgtctagtagtggttgagtttgttgggttcttgtaacgtttcctgattcacatgctcacttgcatgggagggtcatggaaattatacattggatgcactcataatgaaaactcacaatggatttccttaagatttatgaatttctcaaattttagtccagtaaccctaaccctaaagctaaaactggtttaagccaccctcagttgctttacaattgctagggacatgaaactatcccacagcagctgttcatgaatcccctaaaactttaagcgagagaagagggagtgattctccttcggaaaaacattccaaggcctttaatgggcctctggatgactgcctggtgtccacccttgtactaaaccagtttccctgcaacttccacctttggttctagtcaacattaacaccttaccaggaccattcgattgggcaaatgctactatacacttggacaaatccagaggtcaattgtttcccccactggttaggttatgtgccaatcctccacctgtagtcacataaaatgtgacattttaccagcaagaattgtttcaagaacgcaattgtttcaacgaatagctcactctctaaccactaattctttttccacaccttgttagctatgcctttttttac

SEQ ID NO: 8 - DNA, 2884 bp, Homo sapiens
tcactcccaggagttcggcagcttttgcacattttaagatcaactgagagtttataaatatgccccgtttttctatgaccatcgctatgggaagagatgaatgtgttctaacctgtttcccatcaaaacttgtgttctaaccccaaaaggaaaagcagcaataaaaacaaccaaaacattttttaaaaataggttctatagtttcaaaaacaataaaaagaataagagccaagcctggaggtgcgcgcctgtagtcccagctacttaggaggctgaggcaagaggatggcttcagctggggaggttgaggctggagtgcagtggcgcagtctcggctcactgcaacctccgcctcctgagttcaagcgtttctcctgcctcaacctcccgagtagctgggattacaggtgcataccaccacgcctggctaatttttgttttgttttgtttcgtttgtttgtttttttgagagggagtctctctctgtctcccaggctggagtgcagtggtgcaatctcggctcactgcaagctcagccttccaggttcacgccattctcctgcctcagcctcccaggtagctgggactacaggctcctgccaccacgcccagctaattttttttttttttttttttgtatttttagtagagagggggtttcaccgtgttagccaggatggtctcaatctcctgagctcatgatccgcctgccttggcctcccaaagtgctgggattacaggcgtgagccaccactcccggcctcctccagccccatctcttcacatgcttttcccacctcagttatgctggtctcctttctgttcctcaaatatgcccaagtcttccagccccagggcccccgtgctatttcctgcctctccaccttctgcaaagctaaggcccatcttccaggtctcacataaatactgtctttcccgaaagcctcttccaaccatccacaagcaggatcccaaactcctcccattcaacctgacagcctcacatagctcctgtcaccatgtgtaatttttgcttactagcagatcaaagaacagaagcaagccgtttgattgtttctttttgttttgttttgtttttagacagagtctcacgagcctccttacaaaatagaaaagtcaatgggatttcagggaaaatggataatcttcgttgggggcagtcaaggaaggctttgtggaacctttgaattaggtcttgacattatatcttgacagtactttgaataaatacaaataatgttatttttttgttaagactcatgcaaccgcatctatgtaaatgaatccgtacatagtattcattcgagtgtgaaatcagactttgggatgctttaaaatttaacagtcaggaacacttactctattttatggacttaaatttgttgaggtggcagggaacaacttgagtgaagggtgggacatggcagtgtgtatgtgggggaaaaaggtggccagcagataagggaagcaggggacagagtattttgagggattagacctgaccagctataacaggaaatagaggctgtagattgaaggatagctacaatggatgttatggagaaattccaactggggtggaaacatgtagctgcaaaattggaagagcagcttattctaggcagaaaagaagaaagtaaaaggcatctgaggggacactaaattaatgcttactgataagtaaacaagcctctggaagtagaaaggtaaaagcataaattgcttggtcaaccacaaccgcttgggagtgctggaggcttcatgactaaaccaaagtctgtccctgaagctccctcttccggcagaaataaatactgcacactaagctggctgactcctttcattaaaaggtgcttgccaatctctaaacagtttacctgtatgggagtcataattgtaatatcttggtgaggattttgttgtgctttcaggcaaaccataaaaggaacactaatttaaataaatacaaacaatgttattttattcttaagattcaggcaaccacatctatgtaagtgaatccttacatggtattcattcaagtgtgaaaccaaactttaggatgctttaaaatttaacaatcaggaacaagactctgttaaaaaaaaaaaaaaagaaatgttagaactctgtcaaactataaaaatataaagtgaaatagcacagtgcagacagactgtacagaccagtgtgctacctttcatgtaaaggggaattacatatattatatatatgatttttttattatttgtgtatatacagtactcactgtatatgcataaagtctgcaagtacatgctggggggaaggggtggatgggagacaaggatggaagatttttttgttgtttttttttggagaccgagtctcgctctgtcactcaggctggagggcagtggcaccatctcagctcactgcaacctccacctcccaggttcaagagattctcctgcctcagcctcccgagtagctgggactacaggcatccatcaccacgctcagctaatttttgtattttattagagatgaggttttgctatatatatatatatatatatatatgaatatatgaatatatatatatgaatatatgaatatatatatatatatgaatatatgaatatatatatattggccaggctggtctcgaactcctgccctcaggtgatctgcccacctcagcctcccaaagtgctgggattacaggtgtgagtggcctggaagattttttattatatactgtttaaaagtttttaagtagttgaaacacatgaagacatcacctcaaaaagttatattaacaattcaaaaatatgcacattaaggattaatttttttgaaaaatttaaaaattgagaaatat

SEQ ID NO: 9 - DNA, 1501 bp, Homo sapiens
catgggacagtaacacagtaatcatgaagaattataaaaataagtgctggccgggagcagtggctcaagcctataatcccagcactttgggaggccgaggcgggcagatcacaaggtcaggagatcaagaccatcctggctaacacagtgaaaccctgtctctactaaaaatacaaaaaaaattagacgggctttgtagagggcgcctggagtcccagctactcgggagactgaggcaggagaatggtgtgaactcatgaggtggagcttgcagtgagccgagatcacgccactgcactccagcatggacaacagagcgagactccctctcaaaaaaaataaataaataagtgctaaggctgattattttattagccctaagaatccaattaaaatagaaatcttgtatttatgctattctttcaaaatctttatgtaaagcaagcttttaataggatgttataaaaatagattttgctccttgtgttcaagtttctcctcttgaaattgcacattttacattttttaaaaaattaaaattaaaaaacaaaatagtatgatagtgttaatttggcagttccaactttagtaacctatcttacagaaatatgaatagacaaaataaagatgtgtgaggatgtactttgcagcagcattataatagcaaaaacctggaaacaaatattgatggacaggttaagtaaatcataggacattcatacaatggaatactagcaaaaatattaaaaagaatgaggtagatattgatatgctagtatggaaagatgtccataattatctagttccccacctcaaaaaaaaaaaaaaaacctgagaatcattatactgagaatggtccaatttgtgtctgtatgtacataatatgtacataacaaatatagtatatttttacacaggggaaaagtccaaaagaatatcaacctgtaaaaagtagttatcccagctgggtgaggttgctcatgcctgtaatcccagcactttgggaggcagaggcaggcggatcacaaggtcaggagatcgagaccatcctggctaacacagtgaaaccctgtctctactaaaaatacaaaaaattagccaggtatggcgaggtgagcctgtagtcctagttgttggggaggctgaggcaggagaatagcgtgaaccagggaggaggagcttgcagtgagccgagatggtgccactgcactccagcctgggctacacagcgagactccatctcaaaaagaaaaagtagttagttatccctggaaagtaaaattgagtaggaacttaaatgggttactatcacctttgactttataaaggtgcacacaaacacacaaaatgtgtatgtatttaattacaaacagtaagagacctggcatggtgcctcacacctgtaatctcagcactttgggaggcagaggcaggagaatcacttgaggccaggagtttgagaccaacctatgcaacaagcgaaatccaacccccccttttc

SEQ ID NO: 10 - DNA, 1501 bp, Homo sapiens
gttttatggacttaaatttgttgaggtggcagggaacaacttgagtgaagggtgggacatggcagtgtgtatgtgggggaaaaaggtggccagcagataagggaagcaggggacagagtattttgagggattagacctgaccagctataacaggaaatagaggctgtagattgaaggatagctacaatggatgttatggagaaattccaactggggtggaaacatgtagctgcaaaattggaagagcagcttattctaggcagaaaagaagaaagtaaaaggcatctgaggggacactaaattaatgcttactgataagtaaacaagcctctggaagtagaaaggtaaaagcataaattgcttggtcaaccacaaccgcttgggagtgctggaggcttcatgactaaaccaaagtctgtccctgaagctccctcttccggcagaaataaatactgcacactaagctggctgactcctttcattaaaaggtgcttgccaatctctaaacagtttacctgtatgggagtcataattgtaatatcttggtgaggattttgttgtgctttcaggcaaaccataaaaggaacactaatttaaataaatacaaacaatgttattttattcttaagattcaggcaaccacatctatgtaagtgaatccttacatggtattcattcaagtgtgaaaccaaactttaggatgctttaaaatttaacaatcaggaacaagactctgttaaaaaaaaaaaaaaagaaatgttagaactctgtcaaactataaaaatataaagtgaaatagcacagtgcagacagactgtacagaccagtgtgctacctttcatgtaaaggggaattacatatattatatatatgatttttttattatttgtgtatatacagtactcactgtatatgcataaagtctgcaagtacatgctggggggaaggggtggatgggagacaaggatggaagatttttttgttgtttttttttggagaccgagtctcgctctgtcactcaggctggagggcagtggcaccatctcagctcactgcaacctccacctcccaggttcaagagattctcctgcctcagcctcccgagtagctgggactacaggcatccatcaccacgctcagctaatttttgtattttattagagatgaggttttgctatatatatatatatatatatatatgaatatatgaatatatatatatgaatatatgaatatatatatatatatgaatatatgaatatatatatattggccaggctggtctcgaactcctgccctcaggtgatctgcccacctcagcctcccaaagtgctgggattacaggtgtgagtggcctggaagattttttattatatactgtttaaaagtttttaagtagttgaaacacatgaagacatcacctcaaaaagttatattaacaattcaaaaatatgcacattaaggattaatttttttgaaaaatttaaaaattgagaaatat

SEQ ID NO: 11 - DNA, 14 bp, Homo sapiens
gcgctcgctcgctc

SEQ ID NO: 12 - DNA, 6015 bp, Homo sapiens
attgcaaatacacacaattatacataaaggcacagaatacatacagaaccagagctacacggtaacaccctgaagaccgacttcttgttttcctgggggaaggaggttggtgtgtaagtatgtggaaagtgtggggttcagggaccacacctaagagccaccagaactatccctttctatagaaacaggcttcgtggcggatgaagaccccatcttggggttccaccagatattcctactaaagaacatcagctgggtgtggtggctcatgcctgtaatcccagcactttgggaagctgaggcgggtggatcacttgaggtcaggagatcgagaccagcctggccaacatggtgaaaccttgtctctactaaaaatacaaaaattagccaggcgtggagcacgcctgtaatcccagctacttgggaggctgaggtaggagaatcacttgaacctgggaggcggaggttgcagtgagccgagatcacatcactgcactccagcctgggcgacacagtgagactccgtctcaaaaacaaaacaaaaccaaacaaaacaaaacatcagcgatgcaatgatgcttgggtttgcaccaatgatatgcaggcttgctctgcacaacttcagctgacctcctctccaccgggccctcacgctgcctcctcttccctcctctttccagaactattgccactcctccagatatgatgcacaaatgagcagggtcgcagtgggagtgggcgcagtgcgctgatgccacggaggtgttgtgcatgacgtctggacactagactagctgcatgtaatgggaaaagtttgtgttgtaccagcgcatgccttggaaagacttaagtaatgcaaaaggttgtcctttaaaaaaaaaaaaaatctggccggtcgcggcggctcacgcctgtaatcccagcattttgggaggccgaggcagtcggatcacgaggtcaggaattcgagaccagcctggccaacatggtgaaaccccgtctctactaaaaaacaaaaattagccgggcgtggtggagcacgcctgtagtcccagctactcaggaggctgaggcaggagaatcgcttgaacccgggaggcagagcttgcagtgagccgacatcgcgccactgcactccagcctgggcgacagagcaagcctccgtctcaaaaacaacaacaacaacaaaaaaaaacaaaactactgacaagttgctctacttaacccaaagaaagtgaaggagaaagcggctgcctcaccgcctagacattgagtcgccggatgtttcaatgcctcatgatacaataaaaccacaaaaattttcgtaacagcagcagcaacaacaacaacaaaagagaaagagagagggaaagaaacaggcctcgtgggatgcgcagtttacgtctccgcgcaaacccaaggacttcagagtgggtgggaaactcccacagcgcttgggaaacagtctgtagtctctgtcccgattttggcccttttctgtatgatttttatgggactcttcctgtcacaaagtgccagccaccttcccaatcttgagttgggcgcgggatccgtaaggtgaagatcaaggtgtgctcatcgcttgggcccgctgaaaggtgattcgccccccacctgctggaactccttgcccgggaccaccaatcccagcatgccttgagagcgcgcgagggcctgggcggttcccaggaggtccgggtgggcgcaggagaagcgcgggccagtgaaagctctgagagccctgtccctgtggacactgtgtcttgggttcctttactcggtgtggctcagggattaccattagggagtggagtgtggatttctcttgccccgagccctaaatgccttggggccctgccttgcaccccactgtgcttttaggggtgtggccctgtgggctacatttcccagcgtgccctaggatcgtggtcctgaccttttcaccgcaaatttcatttcccagcatgccctgcgaggtcacccagggaagcttggaagtggactgtctttcatggcttctaggttgcggactcagtttcccatggtgccctggtgaacccattcattcattcattccaaaaatatttgcgatcaggttctctcaggttctgttctaagaaccgaggacaagtagtgcacagaagacaaaagatcccgctctcgtggagcttatttctagttaaggggtcaggaaaaaaaccaaaataaataaaacccagctgggcatggtggcttacgctcgtcatcccagcaggattacaggccgaggcgggcggatcatgaggtcaagagatcaagaccatcatggccaacatggtgaaatcccgtctctactaaaaatataaaaattagcagggcggggtggcgcgcgcctgttatcccagctactctggggactgagccagaattgcttgaacctgggaagcggaggttgcagcgagccgatatcgcgccactgaactccagcgtggcgacagagcgagactccgtctcaaaacaaagaaaacaaaataaaacaacaataacaaaacaactctgcctctccccgcactccctcccacgcggctgtccagtcgaattcctaactgccccggggcagtctgctattcatcccctttacccggtgctacacacttcctagtatgccgtggggcacccctccggcctgtagactccatttcccagcattccccggaggaggccctcatctggcgatttccactgggcgcctcggagctgcggacttcccagtgtgcatcggggcacagcgactcctggaagtggccaagggccacttctgctaatggactccatttcccagcgctccccgcgacctgcccagcacaccctggggcagcgccgtgacgtcagcacgccgggcggggaccgggagatccttggggcggtggggggccagcggcagttcccggcggcccccggggcgggcgggcgggcgggtggtggcggcggttggggctcggcgctcgctcgctcgctgggcgggcgggcggtgcgatgtccggagaggatggcccggcggctggcccgggggcggcggcggcggctgcccgggagcggcgacgggagcagctgcggcagtggggggcgcgggcgggcgccgagcctggccccggagagcgccgcgcccgcaccgtccgcttcgagcgcgccgccgagttcctggcggcctgtgcgggcggcgacctggacgaggcgcgtctgatgctgcgcgccgccgaccctggccccggcgccgagctcgaccccgccgcgccgccgcccgcccgcgccgtgctggactccaccaacgccgacggtatcagcgccctgcaccaggtcagcgccccccgcccggcgtctcccggggccaggtccaccctctgctgcgccacctggggcatcctccttccccgttgccagtctcgatccgccccgtcgttcctggccctgggctttgccaccctatgctgacaccccgtcccagtcccccttaccattccccttcgaccaccccacttccgaattggagccgcttcaactggccctgggcttagccactctgtgctgaccactctgccccaggcctccttaccattccccttcgacctactctcttccgcattggagtcgctttaactggccctggctttggcagcctgtgctgacccatgcagtcctccttaccatccctccctcgacttcccctcttccgatgttgagcccctccagccggtcctggactttgtctccttccctgccctgccctctcctgaacctgagccagctcccatagctcagtctggtctatctgcctggccctggccattgtcactttgcgctgccctcctctcgcccccgagtgcccttgctgtgccgccggaactctgccctctaacgctgccgtctctctcctgagtccggaccactttgagctctactggcttctgcgccgcctctggcccactgtttccccttcccaggcaggtcctgctttctctgacctgcattctctcccctgggcctgtgccgctttctgtctgcagcttgtggcctgggtcacctctacggctggcccagatccttccctgccgcctccttcaggttccgtcttcctccactccctcttccccttgctctctgctgtgttgctgcccaaggatgctctttccggagcacttccttctcggcgctgcaccacgtgatgtcctctgagcggatcctccccgtgtctgggtcctctccgggcatctctcctccctcacccaaccccatgccgtcttcactcgctgggttcccttttccttctccttctggggcctgtgccatctctcgtttcttaggatggccttctccgacggatgtctcccttgcgtcccgcctccccttcttgtaggcctgcatcatcaccgtttttctggacaaccccaaagtaccccgtctccctggctttagccacctctccatcctcttgctttctttgcctggacaccccgttctcctgtggattcgggtcacctctcactcctttcatttgggcagctcccctaccccccttacctctctagtctgtgctagctcttccagccccctgtcatggcatcttccaggggtccgagagctcagctagtcttcttcctccaacccgggcccctatgtccacttcaggacagcatgtttgctgcctccagggatcctgtgtccccgagctgggaccaccttatattcccagggccggttaatgtggctctggttctgggtacttttatctgtcccctccaccccacagtggggccactagggacaggattggtgacagaaaagccccatccttaggcctcctccttcctagtctcctgatattgggtctaacccccacctcctgttaggcagattccttatctggtgacacacccccatttcctggagccatctctctccttgccagaacctctaaggtttgcttacgatggagccagagaggatcctgggagggagagcttggcagggggtgggagggaagggggggatgcgtgacctgcccggttctcagtggccaccctgcgctaccctctcccagaacctgagctgctctgacgcggctgtctggtgcgtttcactgatcctggtgctgcagcttccttacacttcccaagaggagaagcagtttggaaaaacaaaatcagaataagttggtcctgagttctaactttggctcttcacctttctagtccccaatttatattgttcctccgtgcgtcagttttacctgtgagataaggccagtagccagccccgtcctggcagggctgtggtgaggaggggggtgtccgtgtggaaaactccctttgtgagaatggtgcgtcctaggtgttcaccaggtcgtggccgcctctactccctttctctttctccatccttctttccttaaagagtccccagtgctatctgggacatattcctccgcccagagcagggtcccgcttccctaaggccctgctctgggcttctgggtttgagtccttggcaagcccaggagaggcgctcaggcttccctgtcccccttcctcgtccaccatctcatgcccctggctctcctgccccttccctacaggggttcctggctctgctcttcagactgagccccgttcccctgcatccccgttcccctgcatcccccttcccctgcatcccccagaggccccaggccacctacttggcctggaccccacgagaggccaccccagccctgtctaccaggctgccttttgggtggattctcctccaactgtggggtgactgcttggcaaactcactcttcggggtatcccaggaggcctggagcattggggtgggctggggttcagagaggagggattcccttctcaggttacgtggccaagaagcaggggagctgggtttgggtcaggtctgggtgtggggtgaccagcttatgctgtttgcccaggacagcctagttttagcgctgaaaccctc